European Patent Specification EP 4 058 035 B1, published September 23, 2026. Title: COMPOSITIONS AND METHODS FOR IMMUNOTHERAPY. Applicant: Ludwig Institute for Cancer Research Ltd. Coukos, George Osorio, de Jesus Corria Zoete, Vincent Irving, Melita. The sequence listing filed with the application follows.

SEQUENCE LISTING (52 sequences)

SEQ ID NO: 1 - protein, 147 aa, Mus musculus
SGWLLEVPNGPWRSLTFYPAWLTVSEGANATFTCSLSNWSEDLMLNWNRLSPSNQTEKQAAFSNGLSQPVQDARFQIIQLPNRHDFHMNILDTRRNDSGIYLCGAISLHPKAKIEESPGAELVVTERILETSTRYPSPSPKPEGRFQ

SEQ ID NO: 2 - protein, 288 aa, Homo sapiens
MQIPQAPWPVVWAVLQLGWRPGWFLDSPDRPWNPPTFSPALLVVTEGDNATFTCSFSNTSESFVLNWYRMSPSNQTDKLAAFPEDRSQPGQDCRFRVTQLPNGRDFHMSVVRARRNDSGTYLCGAISLAPKAQIKESLRAELRVTERRAEVPTAHPSPSPRPAGQFQTLVVGVVGGLLGSLVLLVWVLAVICSRAARGTIGARRTGQPLKEDPSAVPVFSVDYGELDFQWREKTPEPPVPCVPEQTEYATIVFPSGMGTSSPARRGSADGPRSAQPLRPEDGHCSWPL

SEQ ID NO: 3 - protein, 147 aa, Homo sapiens
PGWFLDSPDRPWNPPTFSPALLVVTEGDNATFTCSFSNTSESFVLNWYRMSPSNQTDKLAAFPEDRSQPGQDCRFRVTQLPNGRDFHMSVVRARRNDSGTYLCGAISLAPKAQIKESLRAELRVTERRAEVPTAHPSPSPRPAGQFQ

SEQ ID NO: 4 - protein, 371 aa, Artificial sequence
  Synthetic
PGWFLDSPDRPWNPPTFSPALLVVTEGDNATFTCSFSNTSESFVLNWYRMSPSNQTDKLAAFPEDRSQPGQDCRFRVTQLPNGRDFHMSVVRARRNDSGTYLCGAISLAPKAQIKESLRAELRVTERRAEVPTAHPSPSPRPAGQFQPPCPSCPAPEFLGGPSVFLFPPKPKDTLMISRTPEVTCVVVDVSQEDPEVQFNWYVDGVEVHNAKTKPREEQFNSTYRVVSVLTVLHQDWLNGKEYKCKVSNKGLPSSIEKTISKAKGQPREPQVYTLPPSQEEMTKNQVSLTCLVKGFYPSDIAVEWESNGQPENNYKTTPPVLDSDGSFFLYSRLTVDKSRWQEGNVFSCSVMHEALHNHYTQKSLSLSPGK

SEQ ID NO: 5 - DNA, 1113 bp, Artificial sequence
  Synthetic
cctggctggtttctggacagccctgacagaccctggaatcctccaacattcagccccgctctgctggtggttaccgagggcgataatgccaccttcacctgtagcttcagcaacaccagcgagagcttcgtgctgaactggtacagaatgagccccagcaaccagaccgacaagctggccgcctttcctgaggatagatctcagcccggccaggactgccggttcagagttacacagctgcccaacggccgggacttccacatgtctgtcgtccgggccagaagaaacgacagcggcacatatctgtgcggcgccatttctctggcccctaaggctcagatcaaagagagcctgagagccgagctgagagtgacagaaagacgggccgaagtgcccacagctcacccttcaccttctccaagacctgccggccagtttcagcctccttgtcctagctgtcctgctcctgagtttctcggcggaccctccgtgttcctgtttcctccaaagcctaaggacaccctgatgatcagcagaacccctgaagtgacctgcgtggtggtggacgtgtcccaagaggaccctgaggtgcagttcaattggtacgtggacggcgtggaagtgcacaacgccaagaccaagcctagagaggaacagttcaacagcacctacagagtggtgtccgtgctgaccgtgctgcaccaggattggctgaacggcaaagagtacaagtgcaaggtgtccaacaagggcctgcctagcagcatcgagaaaaccatcagcaaggccaagggccagccaagagaaccccaggtgtacacactgcctccaagccaagaggaaatgaccaagaaccaggtgtccctgacctgcctggtcaagggcttctacccttccgatatcgccgtggaatgggagagcaatggccagcctgagaacaactacaagaccacacctcctgtgctggacagcgacggctcattcttcctgtacagcagactgaccgtggacaagagcagatggcaagagggcaacgtgttcagctgcagcgtgatgcacgaggccctgcacaaccactacacccagaagtccctgagcctgtctcctggcaaa

SEQ ID NO: 6 - protein, 129 aa, Artificial sequence
  Synthetic
MASDSPDRPWNPPTFSPALLVVTEGDNATFTCSFSNTSESFVLNWYRMSPSNQDDRLAAFPEDRSQPGQDARFRVTQLPNGRDFHMSVVRARRNDSGTYFCGAISLAPKAKIKESLRAELRVTERRALE

SEQ ID NO: 7 - protein, 135 aa, Artificial sequence
  Synthetic
MASDSPDRPWNPPTFSPALLVVTEGDNATFTCSFSNTSESFVLNWYRMSPSNQDDRLAAFPEDRSQPGQDARFRVTQLPNGRDFHMSVVRARRNDSGTYFCGAISLAPKAKIKESLRAELRVTERRALEHHHHHH

SEQ ID NO: 8 - protein, 367 aa, Artificial sequence
  Synthetic
DSPDRPWNPPTFSPALLVVTEGDNATFTCSFSNTSESFVLNWYRMSPSNQDDRLAAFPEDRSQPGQDARFRVTQLPNGRDFHMSVVRARRNDSGTYFCGAISLAPKAKIKESLRAELRVTERRAEVPTAHPSPSPRPAGQFQTPPCPSCPAPEFLGGPSVFLFPPKPKDTLMISRTPEVTCVVVDVSQEDPEVQFNWYVDGVEVHNAKTKPREEQFNSTYRVVSVLTVLHQDWLNGKEYKCKVSNKGLPSSIEKTISKAKGQPREPQVYTLPPSQEEMTKNQVSLTCLVKGFYPSDIAVEWESNGQPENNYKTTPPVLDSDGSFFLYSRLTVDKSRWQEGNVFSCSVMHEALHNHYTQKSLSLSLGK

SEQ ID NO: 9 - protein, 129 aa, Artificial sequence
  Synthetic
MASDSPDRPWNPPTFSPALLVVTEGDNATFTCSFSNTSESFVLNWYRMSPSNQVDRLAAFPEDRSQPGQDARFRVTQLPNGRDFHMSVVRARRNDSGTYFCGAISLAPKWKIKESLRAELRVTERRALE

SEQ ID NO: 10 - protein, 135 aa, Artificial sequence
  Synthetic
MASDSPDRPWNPPTFSPALLVVTEGDNATFTCSFSNTSESFVLNWYRMSPSNQVDRLAAFPEDRSQPGQDARFRVTQLPNGRDFHMSVVRARRNDSGTYFCGAISLAPKWKIKESLRAELRVTERRALEHHHHHH

SEQ ID NO: 11 - protein, 367 aa, Artificial sequence
  Synthetic
DSPDRPWNPPTFSPALLVVTEGDNATFTCSFSNTSESFVLNWYRMSPSNQVDRLAAFPEDRSQPGQDARFRVTQLPNGRDFHMSVVRARRNDSGTYFCGAISLAPKWKIKESLRAELRVTERRAEVPTAHPSPSPRPAGQFQTPPCPSCPAPEFLGGPSVFLFPPKPKDTLMISRTPEVTCVVVDVSQEDPEVQFNWYVDGVEVHNAKTKPREEQFNSTYRVVSVLTVLHQDWLNGKEYKCKVSNKGLPSSIEKTISKAKGQPREPQVYTLPPSQEEMTKNQVSLTCLVKGFYPSDIAVEWESNGQPENNYKTTPPVLDSDGSFFLYSRLTVDKSRWQEGNVFSCSVMHEALHNHYTQKSLSLSLGK

SEQ ID NO: 12 - protein, 129 aa, Artificial sequence
  Synthetic
MASDSPDRPWNPPTFSPALLVVTEGDNATFTCSFSNTSESFVLNWYRESPSNQDDRLAAFPEDRSQPGQDARFRVTQLPNGRDFHMSVVRARRNDSGTYFCGAISLAPKAKIKESLRAELRVTERRALE

SEQ ID NO: 13 - protein, 135 aa, Artificial sequence
  Synthetic
MASDSPDRPWNPPTFSPALLVVTEGDNATFTCSFSNTSESFVLNWYRESPSNQDDRLAAFPEDRSQPGQDARFRVTQLPNGRDFHMSVVRARRNDSGTYFCGAISLAPKAKIKESLRAELRVTERRALEHHHHHH

SEQ ID NO: 14 - protein, 370 aa, Artificial sequence
  Synthetic
MASDSPDRPWNPPTFSPALLVVTEGDNATFTCSFSNTSESFVLNWYRESPSNQDDRLAAFPEDRSQPGQDARFRVTQLPNGRDFHMSVVRARRNDSGTYFCGAISLAPKAKIKESLRAELRVTERRAEVPTAHPSPSPRPAGQFQTPPCPSCPAPEFLGGPSVFLFPPKPKDTLMISRTPEVTCVVVDVSQEDPEVQFNWYVDGVEVHNAKTKPREEQFNSTYRVVSVLTVLHQDWLNGKEYKCKVSNKGLPSSIEKTISKAKGQPREPQVYTLPPSQEEMTKNQVSLTCLVKGFYPSDIAVEWESNGQPENNYKTTPPVLDSDGSFFLYSRLTVDKSRWQEGNVFSCSVMHEALHNHYTQKSLSLSLGK

SEQ ID NO: 15 - protein, 129 aa, Artificial sequence
  Synthetic
MASDSPDRPWNPPTFSPALLVVTEGDNATFTCSFSNTSESFVLNWYRESPSNQVDRLAAFPEDRSQPGQDARFRVTQLPNGRDFHMSVVRARRNDSGTYFCGAISLAPKWKIKESLRAELRVTERRALE

SEQ ID NO: 16 - protein, 135 aa, Artificial sequence
  Synthetic
MASDSPDRPWNPPTFSPALLVVTEGDNATFTCSFSNTSESFVLNWYRESPSNQVDRLAAFPEDRSQPGQDARFRVTQLPNGRDFHMSVVRARRNDSGTYFCGAISLAPKWKIKESLRAELRVTERRALEHHHHHH

SEQ ID NO: 17 - protein, 370 aa, Artificial sequence
  Synthetic
MASDSPDRPWNPPTFSPALLVVTEGDNATFTCSFSNTSESFVLNWYRESPSNQVDRLAAFPEDRSQPGQDARFRVTQLPNGRDFHMSVVRARRNDSGTYFCGAISLAPKWKIKESLRAELRVTERRAEVPTAHPSPSPRPAGQFQTPPCPSCPAPEFLGGPSVFLFPPKPKDTLMISRTPEVTCVVVDVSQEDPEVQFNWYVDGVEVHNAKTKPREEQFNSTYRVVSVLTVLHQDWLNGKEYKCKVSNKGLPSSIEKTISKAKGQPREPQVYTLPPSQEEMTKNQVSLTCLVKGFYPSDIAVEWESNGQPENNYKTTPPVLDSDGSFFLYSRLTVDKSRWQEGNVFSCSVMHEALHNHYTQKSLSLSLGK

SEQ ID NO: 18 - protein, 224 aa, Homo sapiens
PPCPSCPAPEFLGGPSVFLFPPKPKDTLMISRTPEVTCVVVDVSQEDPEVQFNWYVDGVEVHNAKTKPREEQFNSTYRVVSVLTVLHQDWLNGKEYKCKVSNKGLPSSIEKTISKAKGQPREPQVYTLPPSQEEMTKNQVSLTCLVKGFYPSDIAVEWESNGQPENNYKTTPPVLDSDGSFFLYSRLTVDKSRWQEGNVFSCSVMHEALHNHYTQKSLSLSPGK

SEQ ID NO: 19 - protein, 327 aa, Homo sapiens
ASTKGPSVFPLAPCSRSTSESTAALGCLVKDYFPEPVTVSWNSGALTSGVHTFPAVLQSSGLYSLSSVVTVPSSSLGTKTYTCNVDHKPSNTKVDKRVESKYGPPCPSCPAPEFLGGPSVFLFPPKPKDTLMISRTPEVTCVVVDVSQEDPEVQFNWYVDGVEVHNAKTKPREEQFNSTYRVVSVLTVLHQDWLNGKEYKCKVSNKGLPSSIEKTISKAKGQPREPQVYTLPPSQEEMTKNQVSLTCLVKGFYPSDIAVEWESNGQPENNYKTTPPVLDSDGSFFLYSRLTVDKSRWQEGNVFSCSVMHEALHNHYTQKSLSLSLGK

SEQ ID NO: 20 - protein, 108 aa, Mus musculus
DVQMIQSPSSLSASLGDIVTMTCQASQGTSINLNWFQQKPGKAPKLLIYGASILEDGVPSRFSGSRYGTDFTLTISSLEDEDMATYFCLQHSYLPYTFGGGTKLEIKR

SEQ ID NO: 21 - protein, 153 aa, Homo sapiens
MYRMQLLSCIALSLALVTNSAPTSSSTKKTQLQLEHLLLDLQMILNGINNYKNPKLTRMLTFKFYMPKKATELKHLQCLEEELKPLEEVLNLAQSKNFHLRPRDLISNINVIVLELKGSETTFMCEYADETATIVEFLNRWITFCQSIISTLT

SEQ ID NO: 22 - protein, 133 aa, Artificial sequence [sequence omitted]

SEQ ID NO: 23 - protein, 133 aa, Artificial sequence
  Synthetic
APTSSSTKKTQLQLEHLLLDLQMILNGINNYKNPKLTAMLTAKFAMPKKATELKHLQCLEEALKPLEEVLNLAQSKNFHLRPRDLISNINVIVLELKGSETTFMCEYADETATIVEFLNRWITFSQSIISTLT

SEQ ID NO: 24 - DNA, 402 bp, Artificial sequence
  Synthetic
gcccctaccagcagcagcaccaaaaagacacagctgcaactggaacacctcctgctggacctgcagatgatcctgaacggcatcaacaactacaagaaccccaagctgaccgccatgctgacagccaagttcgccatgcctaagaaggccaccgagctgaagcacctccagtgcctggaagaggccctgaagcctctggaagaagtgctgaatctggcccagagcaagaacttccacctgaggcctagggacctgatcagcaacatcaacgtgatcgtgctggaactgaagggcagcgagacaaccttcatgtgcgagtacgccgacgagacagctaccatcgtggaatttctgaaccggtggatcaccttcagccagagcatcatcagcaccctgacctga

SEQ ID NO: 25 - protein, 159 aa, Homo sapiens
SITGISPITEYLASLSTYNDQSITFALEDESYEIYVEDLKKDEKKDKVLLSYYESQHPSNESGDGVDGKMLMVTLSPTKDFWLHANNKEHSVELHKCEKPLPDQAFFVLHNMHSNCVSFECKTDPGVFIGVKDNHLALIKVDSSENLCTENILFKLSET

SEQ ID NO: 26 - DNA, 477 bp, Homo sapiens
agcatcaccggcatcagccccatcacagagtatctggccagcctgagcacctacaacgaccagagcatcacattcgccctggaagatgagagctacgagatctacgtggaagatctgaagaaggacgagaagaaagacaaggtgctgctgagctactacgagtctcagcaccccagcaatgagtctggcgacggcgtggacggaaagatgctgatggttacactgagccccaccaaggatttctggctgcacgccaacaacaaagagcacagcgtcgagctgcacaagtgcgagaagcctctgcctgaccaggccttcttcgtgctgcacaacatgcacagcaactgcgtgtccttcgagtgcaagaccgatcctggcgtgttcatcggcgtgaaggacaaccatctggccctgatcaaggtggacagcagcgagaatctgtgcaccgagaacatcctgttcaagctgagcgagaca

SEQ ID NO: 27 - protein, 158 aa, Mus musculus
SIQGTSLLTQSPASLSTYNDQSVSFVLENGCYVINVDDSGKDQEQDQVLLRYYESPCPASQSGDGVDGKKLMVNMSPIKDTDIWLHANDKDYSVELQRGDVSPPEQAFFVLHKKSSDFVSFECKNLPGTYIGVKDNQLALVEEKDESCNNIMFKLSKI

SEQ ID NO: 28 - protein, 240 aa, Homo sapiens
MEESVVRPSVFVVDGQTDIPFTRLGRSHRRQSCSVARVGLGLLLLLMGAGLAVQGWFLLQLHWRLGEMVTRLPDGPAGSWEQLIQERRSHEVNPAAHLTGANSSLTGSGGPLLWETQLGLAFLRGLSYHDGALVVTKAGYYYIYSKVQLGGVGCPLGLASTITHGLYKRTPRYPEELELLVSQQSPCGRATSSSRVWWDSSFLGGVVHLEAGEKVVVRVLDERLVRLRDGTRSYFGAFMV

SEQ ID NO: 29 - protein, 167 aa, Homo sapiens
DGPAGSWEQLIQERRSHEVNPAAHLTGANSSLTGSGGPLLWETQLGLAFLRGLSYHDGALVVTKAGYYYIYSKVQLGGVGCPLGLASTITHGLYKRTPRYPEELELLVSQQSPCGRATSSSRVWWDSSFLGGVVHLEAGEKVVVRVLDERLVRLRDGTRSYFGAFMV

SEQ ID NO: 30 - DNA, 501 bp, Homo sapiens
gatggacctgccggatcttgggagcagctgatccaagagcggagaagccacgaagtgaaccctgccgcacatctgacaggcgccaattctagcctgacaggctctggtggacccctgctgtgggaaactcaactgggactcgccttcctgagaggcctgagctatcatgatggcgccctggtggttaccaaggccggctactactacatctacagcaaggtgcagctcggcggcgtgggatgtcctcttggactggcctctacaatcacccacggcctgtacaagcggacccctagataccccgaggaactggaactgctggtgtcccagcagagcccttgtggcagagccacaagcagcagcagagtttggtgggacagcagctttctcggcggagtggtgcatctggaagccggcgaaaaggtggtcgtcagagtgctggatgagagactcgtgcggctgagagatggcaccagaagctacttcggcgccttcatggtt

SEQ ID NO: 31 - protein, 168 aa, Mus musculus
DGGKGSWEKLIQDQRSHQANPAAHLTGANASLIGIGGPLLWETRLGLAFLRGLTYHDGALVTMEPGYYYVYSKVQLSGVGCPQGLANGLPITHGLYKRTSRYPKELELLVSRRSPCGRANSSRVWWDSSFLGGVVHLEAGEEVVVRVPGNRLVRPRDGTRSYFGAFMV

SEQ ID NO: 32 - protein, 261 aa, Homo sapiens
MIETYNQTSPRSAATGLPISMKIFMYLLTVFLITQMIGSALFAVYLHRRLDKIEDERNLHEDFVFMKTIQRCNTGERSLSLLNCEEIKSQFEGFVKDIMLNKEETKKENSFEMQKGDQNPQIAAHVISEASSKTTSVLQWAEKGYYTMSNNLVTLENGKQLTVKRQGLYYIYAQVTFCSNREASSQAPFIASLCLKSPGRFERILLRAANTHSSAKPCGQQSIHLGGVFELQPGASVFVNVTDPSQVSHGTGFTSFGLLKL

SEQ ID NO: 33 - protein, 149 aa, Mus musculus
MQRGDEDPQIAAHVVSEANSNAASVLQWAKKGYYTMKSNLVMLENGKQLTVKREGLYYVYTQVTFCSNREPSSQRPFIVGLWLKPSSGSERILLKAANTHSSSQLCEQQSVHLGGVFELQAGASVFVNVTEASQVIHRVGFSSFGLLKL

SEQ ID NO: 34 - protein, 149 aa, Homo sapiens
MQKGDQNPQIAAHVISEASSKTTSVLQWAEKGYYTMSNNLVTLENGKQLTVKRQGLYYIYAQVTFCSNREASSQAPFIASLCLKSPGRFERILLRAANTHSSAKPCGQQSIHLGGVFELQPGASVFVNVTDPSQVSHGTGFTSFGLLKL

SEQ ID NO: 35 - DNA, 447 bp, Homo sapiens
atgcagaagggcgaccagaatcctcagatcgccgctcacgtgatcagcgaggccagcagcaagacaacaagcgtgctgcagtgggccgagaagggctactacaccatgagcaacaacctggtcaccctggaaaacggcaagcagctgaccgtgaagagacagggcctgtactacatctacgcccaagtgaccttctgcagcaacagagaggccagctctcaggccccttttatcgccagcctgtgcctgaagtcccctggcagattcgagcggattctgctgagagccgccaacacacacagcagcgccaaaccttgtggccagcagtctattcacctcggcggagtgtttgagctgcagcctggcgcaagcgtgttcgtgaatgtgacagaccctagccaggtgtcccacggcaccggctttacatctttcggcctgctgaagctg

SEQ ID NO: 36 - protein, 216 aa, Artificial sequence
  Synthetic
MGTNKCLLQIALLLCFSTTALSRMKQIEDKIEEILSKIYHIENEIARIKKLIGEVGGGSGGGSGGGSMQKGDQNPQIAAHVISEASSKTTSVLQWAEKGYYTMSNNLVTLENGKQLTVKRQGLYYIYAQVTFCSNREASSQAPFIASLCLKSPGRFERILLRAANTHSSAKPCGQQSIHLGGVFELQPGASVFVNVTDPSQVSHGTGFTSFGLLKL

SEQ ID NO: 37 - DNA, 651 bp, Artificial sequence
  Synthetic
atgggaacaaacaaatgcctgctgcagatcgccctgctgctgtgctttagcacaacagccctgagccggatgaagcagatcgaggacaagatcgaagagatcctgagcaagatctaccacatcgagaacgagatcgcccggatcaagaaactgatcggcgaagtcggcggaggctctggtggtggatctggcggaggatctatgcagaaaggcgaccagaatcctcagatcgccgctcacgtgatcagcgaggccagcagcaagacaacaagcgtgctgcagtgggccgagaagggctactacaccatgagcaacaacctggtcaccctggaaaacggcaagcagctgaccgtgaagagacagggcctgtactacatctacgcccaagtgaccttctgcagcaacagagaggccagctctcaggccccttttatcgccagcctgtgcctgaagtcccctggcagattcgagcggattctgctgagagccgccaacacacacagcagcgccaaaccttgtggccagcagtctattcacctcggcggagtgtttgagctgcagcctggcgcaagcgtgttcgtgaatgtgacagaccctagccaggtgtcccacggcaccggctttacatctttcggcctgctgaagctctga

SEQ ID NO: 38 - protein, 261 aa, Homo sapiens; identical to SEQ ID NO: 32

SEQ ID NO: 39 - protein, 182 aa, Mus musculus
MNNRWILHAAFLLCFSTTALSINYKQLQLQERTNIRKCQELLEQLNGKINLTYRADFKIPMEMTEKMQKSYTAFAIQEMLQNVFLVFRNNFSSTGWNETIVVRLLDELHQQTVFLKTVLEEKQEERLTWEMSSTALHLKSYYWRVQRYLKLMKYNSYAWMVVRAEIFRNFLIIRRLTRNFQN

SEQ ID NO: 40 - protein, 357 aa, Homo sapiens
MLLLVTSLLLCELPHPAFLLIPRKVCNGIGIGEFKDSLSINATNIKHFKNCTSISGDLHILPVAFRGDSFTHTPPLDPQELDILKTVKEITGFLLIQAWPENRTDLHAFENLEIIRGRTKQHGQFSLAVVSLNITSLGLRSLKEISDGDVIISGNKNLCYANTINWKKLFGTSGQKTKIISNRGENSCKATGQVCHALCSPEGCWGPEPRDCVSCRNVSRGRECVDKCNLLEGEPREFVENSECIQCHPECLPQAMNITCTGRGPDNCIQCAHYIDGPHCVKTCPAGVMGENNTLVWKYADAGHVCHLCHPNCTYGCTGPGLEGCPTNGPKIPSIATGMVGALLLLLVVALGIGLFM

SEQ ID NO: 41 - DNA, 1074 bp, Homo sapiens
atgcttctgctggttacatctctgctgctgtgcgagctgccccatcctgcctttctgctgatccccagaaaagtgtgcaacggcatcggcatcggagagttcaaggacagcctgagcatcaacgccaccaacatcaagcacttcaagaactgcaccagcatcagcggcgacctgcacattctgcctgtggcctttagaggcgacagcttcacccacacacctccactcgatccccaagagctggacatcctgaaaaccgtgaaagagatcaccggatttctgttgatccaggcttggcccgagaaccggacagatctgcacgccttcgagaacctggaaatcatcagaggccggaccaagcagcacggccagttttctctggctgtggtgtccctgaacatcaccagcctgggcctgagaagcctgaaagaaatcagcgacggcgacgtgatcatctccggcaacaagaacctgtgctacgccaacaccatcaactggaagaagctgttcggcaccagcggccagaaaacaaagatcatcagcaaccggggcgagaacagctgcaaggctacaggccaagtgtgccacgctctgtgtagccctgaaggctgttggggacccgagcctagagattgcgtgtcctgcagaaacgtgtcccggggcagagaatgcgtggacaagtgcaatctgctggaaggcgagccccgcgagttcgtggaaaacagcgagtgcatccagtgtcaccccgagtgtctgccccaggccatgaacattacctgtaccggcagaggccccgacaactgtattcagtgcgcccactacatcgacggccctcactgcgtgaaaacatgtcctgctggcgtgatgggagagaacaacaccctcgtgtggaagtatgccgacgccggacatgtgtgccacctgtgtcaccctaattgcacctacggctgtacaggccctggcctggaaggctgtccaacaaacggacctaagatcccctctatcgccaccggcatggttggagccctgctgctgcttctggttgtggcccttggcatcggcctgtttatgtag

SEQ ID NO: 42 - protein, 752 aa, Artificial sequence
  Synthetic
DSPDRPWNPPTFSPALLVVTEGDNATFTCSFSNTSESFVLNWYRMSPSNQDDRLAAFPEDRSQPGQDARFRVTQLPNGRDFHMSVVRARRNDSGTYFCGAISLAPKAKIKESLRAELRVTERRAEVPTAHPSPSPRPAGQFQTPPCPSCPAPEFLGGPSVFLFPPKPKDTLMISRTPEVTCVVVDVSQEDPEVQFNWYVDGVEVHNAKTKPREEQFNSTYRVVSVLTVLHQDWLNGKEYKCKVSNKGLPSSIEKTISKAKGQPREPQVYTLPPSQEEMTKNQVSLTCLVKGFYPSDIAVEWESNGQPENNYKTTPPVLDSDGSFFLYSRLTVDKSRWQEGNVFSCSVMHEALHNHYTQKSLSLSLGKASRKRRSGSGEGRGSLLTCGDVEENPGPMLLLVTSLLLCELPHPAFLLIPRKVCNGIGIGEFKDSLSINATNIKHFKNCTSISGDLHILPVAFRGDSFTHTPPLDPQELDILKTVKEITGFLLIQAWPENRTDLHAFENLEIIRGRTKQHGQFSLAVVSLNITSLGLRSLKEISDGDVIISGNKNLCYANTINWKKLFGTSGQKTKIISNRGENSCKATGQVCHALCSPEGCWGPEPRDCVSCRNVSRGRECVDKCNLLEGEPREFVENSECIQCHPECLPQAMNITCTGRGPDNCIQCAHYIDGPHCVKTCPAGVMGENNTLVWKYADAGHVCHLCHPNCTYGCTGPGLEGCPTNGPKIPSIATGMVGALLLLLVVALGIGLFM

SEQ ID NO: 43 - DNA, 2259 bp, Artificial sequence
  Synthetic
gacagccctgacagaccctggaatcctccaacattcagccccgctctgctggtggttaccgagggcgataatgccaccttcacctgtagcttcagcaacaccagcgagagcttcgtgctgaactggtacagaatgagccccagcaaccaggacgacagactggccgcctttcctgaggatagatctcagcccggccaggacgcccggttcagagttacacagctgcccaacggccgggacttccacatgtctgtcgtccgggccagaagaaacgacagcggcacatatttttgcggcgccatttctctggcccctaaggctaaaatcaaagagagcctgagagccgagctgagagtgacagaaagacgggccgaagtgcccacagctcacccttcaccttctccaagacctgccggccagtttcagactcctccttgtcctagctgtcctgctcctgagtttctcggcggaccctccgtgttcctgtttcctccaaagcctaaggacaccctgatgatcagcagaacccctgaagtgacctgcgtggtggtggacgtgtcccaagaggaccctgaggtgcagttcaattggtacgtggacggcgtggaagtgcacaacgccaagaccaagcctagagaggaacagttcaacagcacctacagagtggtgtccgtgctgaccgtgctgcaccaggattggctgaacggcaaagagtacaagtgcaaggtgtccaacaagggcctgcctagcagcatcgagaaaaccatcagcaaggccaagggccagccaagagaaccccaggtgtacacactgcctccaagccaagaggaaatgaccaagaaccaggtgtccctgacctgcctggtcaagggcttctacccttccgatatcgccgtggaatgggagagcaatggccagcctgagaacaactacaagaccacacctcctgtgctggacagcgacggctcattcttcctgtacagcagactgaccgtggacaagagcagatggcaagagggcaacgtgttcagctgcagcgtgatgcacgaggccctgcacaaccactacacccagaagtccctgagcctgtctctgggcaaagccagccggaagagaagatctggatctggcgaaggcagaggctccctgctgacttgcggagatgtggaagagaaccccggacctatgcttctgctggttacatctctgctgctgtgcgagctgccccatcctgcctttctgctgatccccagaaaagtgtgcaacggcatcggcatcggagagttcaaggacagcctgagcatcaacgccaccaacatcaagcacttcaagaactgcaccagcatcagcggcgacctgcacattctgcctgtggcctttagaggcgacagcttcacccacacacctccactcgatccccaagagctggacatcctgaaaaccgtgaaagagatcaccggatttctgttgatccaggcttggcccgagaaccggacagatctgcacgccttcgagaacctggaaatcatcagaggccggaccaagcagcacggccagttttctctggctgtggtgtccctgaacatcaccagcctgggcctgagaagcctgaaagaaatcagcgacggcgacgtgatcatctccggcaacaagaacctgtgctacgccaacaccatcaactggaagaagctgttcggcaccagcggccagaaaacaaagatcatcagcaaccggggcgagaacagctgcaaggctacaggccaagtgtgccacgctctgtgtagccctgaaggctgttggggacccgagcctagagattgcgtgtcctgcagaaacgtgtcccggggcagagaatgcgtggacaagtgcaatctgctggaaggcgagccccgcgagttcgtggaaaacagcgagtgcatccagtgtcaccccgagtgtctgccccaggccatgaacattacctgtaccggcagaggccccgacaactgtattcagtgcgcccactacatcgacggccctcactgcgtgaaaacatgtcctgctggcgtgatgggagagaacaacaccctcgtgtggaagtatgccgacgccggacatgtgtgccacctgtgtcaccctaattgcacctacggctgtacaggccctggcctggaaggctgtccaacaaacggacctaagatcccctctatcgccaccggcatggttggagccctgctgctgcttctggttgtggcccttggcatcggcctgtttatgtag

SEQ ID NO: 44 - protein, 732 aa, Artificial sequence
  Synthetic
DSPDRPWNPPTFSPALLVVTEGDNATFTCSFSNTSESFVLNWYRMSPSNQVDRLAAFPEDRSQPGQDARFRVTQLPNGRDFHMSVVRARRNDSGTYFCGAISLAPKWKIKESLRAELRVTERRPPCPSCPAPEFLGGPSVFLFPPKPKDTLMISRTPEVTCVVVDVSQEDPEVQFNWYVDGVEVHNAKTKPREEQFNSTYRVVSVLTVLHQDWLNGKEYKCKVSNKGLPSSIEKTISKAKGQPREPQVYTLPPSQEEMTKNQVSLTCLVKGFYPSDIAVEWESNGQPENNYKTTPPVLDSDGSFFLYSRLTVDKSRWQEGNVFSCSVMHEALHNHYTQKSLSLSLGKASRKRRSGSGEGRGSLLTCGDVEENPGPMLLLVTSLLLCELPHPAFLLIPRKVCNGIGIGEFKDSLSINATNIKHFKNCTSISGDLHILPVAFRGDSFTHTPPLDPQELDILKTVKEITGFLLIQAWPENRTDLHAFENLEIIRGRTKQHGQFSLAVVSLNITSLGLRSLKEISDGDVIISGNKNLCYANTINWKKLFGTSGQKTKIISNRGENSCKATGQVCHALCSPEGCWGPEPRDCVSCRNVSRGRECVDKCNLLEGEPREFVENSECIQCHPECLPQAMNITCTGRGPDNCIQCAHYIDGPHCVKTCPAGVMGENNTLVWKYADAGHVCHLCHPNCTYGCTGPGLEGCPTNGPKIPSIATGMVGALLLLLVVALGIGLFM

SEQ ID NO: 45 - protein, 675 aa, Homo sapiens
MLLLVTSLLLCELPHPAFLLIPTQVCTGTDMKLRLPASPETHLDMLRHLYQGCQVVQGNLELTYLPTNASLSFLQDIQEVQGYVLIAHNQVRQVPLQRLRIVRGTQLFEDNYALAVLDNGDPLNNTTPVTGASPGGLRELQLRSLTEILKGGVLIQRNPQLCYQDTILWKDIFHKNNQLALTLIDTNRSRACHPCSPMCKGSRCWGESSEDCQSLTRTVCAGGCARCKGPLPTDCCHEQCAAGCTGPKHSDCLACLHFNHSGICELHCPALVTYNTDTFESMPNPEGRYTFGASCVTACPYNYLSTDVGSCTLVCPLHNQEVTAEDGTQRCEKCSKPCARVCYGLGMEHLREVRAVTSANIQEFAGCKKIFGSLAFLPESFDGDPASNTAPLQPEQLQVFETLEEITGYLYISAWPDSLPDLSVFQNLQVIRGRILHNGAYSLTLQGLGISWLGLRSLRELGSGLALIHHNTHLCFVHTVPWDQLFRNPHQALLHTANRPEDECVGEGLACHQLCARGHCWGPGPTQCVNCSQFLRGQECVEECRVLQGLPREYVNARHCLPCHPECQPQNGSVTCFGPEADQCVACAHYKDPPFCVARCPSGVKPDLSYMPIWKFPDEEGACQPCPINCTHSCVDLDDKGCPAEQRASPLTSIISAVVGILLVVVLGVVFGILI

SEQ ID NO: 46 - DNA, 2028 bp, Homo sapiens
atgcttctgctggttacatctctgctgctgtgcgagctgccccatcctgcctttctgctgatccccacacaagtgtgcaccggcaccgacatgaagctgagactgcctgcctctcctgagacacacctggacatgctgagacacctgtaccagggctgtcaggtggtgcagggcaatctggaactgacctacctgcctaccaacgccagcctgagctttctgcaggacatccaagaggtgcagggatacgtgctgattgcccacaatcaagtgcgccaggtgccactgcagcggctgagaatcgttagaggcacccagctgttcgaggacaactatgccctggccgtgctggacaatggcgaccctctgaacaacaccacacctgtgacaggcgcttctcctggcggactgagagaactgcagctgagaagcctgaccgagatcctgaaaggcggcgtgctgatccagagaaaccctcagctgtgctaccaggacaccatcctgtggaaggacatcttccacaagaacaaccagctggccctgacactgatcgacaccaacagaagcagagcctgccatccttgcagccccatgtgcaagggctctagatgttggggcgagagcagcgaggattgccagagcctgaccagaacagtgtgtgccggcggatgtgccagatgcaaaggacctctgcctaccgactgctgccacgagcaatgtgccgctggatgtacaggccccaagcactctgattgcctggcctgcctgcacttcaaccactctggaatctgcgaactgcactgccccgctctggtcacctacaacaccgataccttcgagagcatgcccaatcctgagggcagatacaccttcggcgccagctgtgtgacagcctgtccttacaactacctgagcaccgacgtgggcagctgtacccttgtgtgccctctgcataatcaagaagtgaccgccgaggacggcacccagagatgcgagaagtgtagcaagccttgcgccagagtgtgttacggcctcggcatggaacacctgagagaagtgcgggccgtgaccagcgccaatatccaagaatttgccggctgcaagaagatctttggcagcctcgccttcctgcctgagagcttcgatggcgatcctgccagcaatactgcccctctgcagcctgaacagctccaggtgttcgagacactggaagagatcaccggctacctgtatatcagcgcctggccagacagcctgcctgacctgtccgtgttccagaacctgcaagtgatccggggcagaatcctgcacaacggcgcctattctctgaccctgcaaggcctgggaatcagctggctgggactgagatccctgagagagcttggatctggcctggctctgatccaccacaatacccacctgtgcttcgtgcacaccgtgccttgggaccagctgtttcggaatcctcatcaggccctgctgcacaccgccaacagacctgaggatgagtgtgttggcgaaggcctggcttgtcaccagctctgtgctagaggacactgttggggccctggacctacacagtgcgtgaactgtagccagttcctgcggggccaagagtgcgtggaagagtgtagagttctgcagggactgccccgggaatacgtgaacgccagacactgtctgccttgtcaccctgagtgccagcctcagaatggcagcgtgacctgttttggccctgaggccgatcagtgcgtggcctgtgctcactacaaggaccctccattctgcgtggccagatgtcctagcggcgtgaagcctgatctgagctacatgcccatctggaagttccccgatgaggaaggcgcttgccagccttgtcctatcaactgcacccacagctgcgtggacctggacgataagggatgtccagccgagcagagagcctctccactgacctctatcatctctgccgtcgtgggcatcctgctggtggtggttctgggcgttgtgttcggcatcctgatttga

SEQ ID NO: 47 - protein, 1070 aa, Artificial sequence
  Synthetic
DSPDRPWNPPTFSPALLVVTEGDNATFTCSFSNTSESFVLNWYRMSPSNQDDRLAAFPEDRSQPGQDARFRVTQLPNGRDFHMSVVRARRNDSGTYFCGAISLAPKAKIKESLRAELRVTERRAEVPTAHPSPSPRPAGQFQTPPCPSCPAPEFLGGPSVFLFPPKPKDTLMISRTPEVTCVVVDVSQEDPEVQFNWYVDGVEVHNAKTKPREEQFNSTYRVVSVLTVLHQDWLNGKEYKCKVSNKGLPSSIEKTISKAKGQPREPQVYTLPPSQEEMTKNQVSLTCLVKGFYPSDIAVEWESNGQPENNYKTTPPVLDSDGSFFLYSRLTVDKSRWQEGNVFSCSVMHEALHNHYTQKSLSLSLGKASRKRRSGSGEGRGSLLTCGDVEENPGPMLLLVTSLLLCELPHPAFLLIPTQVCTGTDMKLRLPASPETHLDMLRHLYQGCQVVQGNLELTYLPTNASLSFLQDIQEVQGYVLIAHNQVRQVPLQRLRIVRGTQLFEDNYALAVLDNGDPLNNTTPVTGASPGGLRELQLRSLTEILKGGVLIQRNPQLCYQDTILWKDIFHKNNQLALTLIDTNRSRACHPCSPMCKGSRCWGESSEDCQSLTRTVCAGGCARCKGPLPTDCCHEQCAAGCTGPKHSDCLACLHFNHSGICELHCPALVTYNTDTFESMPNPEGRYTFGASCVTACPYNYLSTDVGSCTLVCPLHNQEVTAEDGTQRCEKCSKPCARVCYGLGMEHLREVRAVTSANIQEFAGCKKIFGSLAFLPESFDGDPASNTAPLQPEQLQVFETLEEITGYLYISAWPDSLPDLSVFQNLQVIRGRILHNGAYSLTLQGLGISWLGLRSLRELGSGLALIHHNTHLCFVHTVPWDQLFRNPHQALLHTANRPEDECVGEGLACHQLCARGHCWGPGPTQCVNCSQFLRGQECVEECRVLQGLPREYVNARHCLPCHPECQPQNGSVTCFGPEADQCVACAHYKDPPFCVARCPSGVKPDLSYMPIWKFPDEEGACQPCPINCTHSCVDLDDKGCPAEQRASPLTSIISAVVGILLVVVLGVVFGILI

SEQ ID NO: 48 - protein, 1050 aa, Artificial sequence
  Synthetic
DSPDRPWNPPTFSPALLVVTEGDNATFTCSFSNTSESFVLNWYRMSPSNQVDRLAAFPEDRSQPGQDARFRVTQLPNGRDFHMSVVRARRNDSGTYFCGAISLAPKWKIKESLRAELRVTERRPPCPSCPAPEFLGGPSVFLFPPKPKDTLMISRTPEVTCVVVDVSQEDPEVQFNWYVDGVEVHNAKTKPREEQFNSTYRVVSVLTVLHQDWLNGKEYKCKVSNKGLPSSIEKTISKAKGQPREPQVYTLPPSQEEMTKNQVSLTCLVKGFYPSDIAVEWESNGQPENNYKTTPPVLDSDGSFFLYSRLTVDKSRWQEGNVFSCSVMHEALHNHYTQKSLSLSLGKASRKRRSGSGEGRGSLLTCGDVEENPGPMLLLVTSLLLCELPHPAFLLIPTQVCTGTDMKLRLPASPETHLDMLRHLYQGCQVVQGNLELTYLPTNASLSFLQDIQEVQGYVLIAHNQVRQVPLQRLRIVRGTQLFEDNYALAVLDNGDPLNNTTPVTGASPGGLRELQLRSLTEILKGGVLIQRNPQLCYQDTILWKDIFHKNNQLALTLIDTNRSRACHPCSPMCKGSRCWGESSEDCQSLTRTVCAGGCARCKGPLPTDCCHEQCAAGCTGPKHSDCLACLHFNHSGICELHCPALVTYNTDTFESMPNPEGRYTFGASCVTACPYNYLSTDVGSCTLVCPLHNQEVTAEDGTQRCEKCSKPCARVCYGLGMEHLREVRAVTSANIQEFAGCKKIFGSLAFLPESFDGDPASNTAPLQPEQLQVFETLEEITGYLYISAWPDSLPDLSVFQNLQVIRGRILHNGAYSLTLQGLGISWLGLRSLRELGSGLALIHHNTHLCFVHTVPWDQLFRNPHQALLHTANRPEDECVGEGLACHQLCARGHCWGPGPTQCVNCSQFLRGQECVEECRVLQGLPREYVNARHCLPCHPECQPQNGSVTCFGPEADQCVACAHYKDPPFCVARCPSGVKPDLSYMPIWKFPDEEGACQPCPINCTHSCVDLDDKGCPAEQRASPLTSIISAVVGILLVVVLGVVFGILI

SEQ ID NO: 49 - protein, 297 aa, Homo sapiens
MTTPRNSVNGTFPAEPMKGPIAMQSGPKPLFRRMSSLVGPTQSFFMRESKTLGAVQIMNGLFHIALGGLLMIPAGIYAPICVTVWYPLWGGIMYIISGSLLAATEKNSRKCLVKGKMIMNSLSLFAAISGMILSIMDILNIKISHFLKMESLNFIRAHTPYINIYNCEPANPSEKNSPSTQYCYSIQSLFLGILSVMLIFAFFQELVIAGIVENEWKRTCSRPKSNIVLLSAEEKKEQTIEIKEEVVGLTETSSQPKNEEDIEIIPIQEEEEEETETNFPEPPQDQESSPIENDSSP

SEQ ID NO: 50 - DNA, 894 bp, Homo sapiens
atgacaacacctagaaatagcgtgaacggcacattccccgccgagcctatgaagggacctatcgccatgcagagcggccccaagcctctgtttagacggatgtctagcctcgtgggccccacacagagctttttcatgagagagagcaagaccctgggcgccgtgcagatcatgaacggcctgtttcacattgccctcggcggcctgctgatgatccctgccggaatctatgcccctatctgcgtgaccgtgtggtatcctctgtggggcggcatcatgtacatcatctctggatctctgctggccgccaccgagaagaacagcagaaagtgtctggtcaagggcaagatgatcatgaatagcctgagcctgttcgccgccatcagcggcatgatcctgagcatcatggatatcctgaatatcaagatcagccacttcctgaagatggaaagcctgaacttcatcagggcccacacaccttacatcaacatctacaactgcgagcccgccaatcctagcgagaagaatagccccagcacacagtactgctactctatccagagcctgtttctgggcatcctgagcgtgatgctgatcttcgcattcttccaagagctggttatcgccggcatcgtggaaaacgagtggaagcggacctgcagcagacccaagagcaacatcgtgctgctgagcgccgaggaaaagaaagagcagaccatcgagatcaaagaggaagtcgtcggcctgaccgagacaagcagccagcctaagaacgaagaggacattgagatcatccccatccaagaagaggaagaagaagagactgagacaaacttccccgagcctcctcaggaccaagagagcagccccattgagaacgacagcagcccttga

SEQ ID NO: 51 - protein, 692 aa, Artificial sequence
  Synthetic
DSPDRPWNPPTFSPALLVVTEGDNATFTCSFSNTSESFVLNWYRMSPSNQDDRLAAFPEDRSQPGQDARFRVTQLPNGRDFHMSVVRARRNDSGTYFCGAISLAPKAKIKESLRAELRVTERRAEVPTAHPSPSPRPAGQFQTPPCPSCPAPEFLGGPSVFLFPPKPKDTLMISRTPEVTCVVVDVSQEDPEVQFNWYVDGVEVHNAKTKPREEQFNSTYRVVSVLTVLHQDWLNGKEYKCKVSNKGLPSSIEKTISKAKGQPREPQVYTLPPSQEEMTKNQVSLTCLVKGFYPSDIAVEWESNGQPENNYKTTPPVLDSDGSFFLYSRLTVDKSRWQEGNVFSCSVMHEALHNHYTQKSLSLSLGKASRKRRSGSGEGRGSLLTCGDVEENPGPMTTPRNSVNGTFPAEPMKGPIAMQSGPKPLFRRMSSLVGPTQSFFMRESKTLGAVQIMNGLFHIALGGLLMIPAGIYAPICVTVWYPLWGGIMYIISGSLLAATEKNSRKCLVKGKMIMNSLSLFAAISGMILSIMDILNIKISHFLKMESLNFIRAHTPYINIYNCEPANPSEKNSPSTQYCYSIQSLFLGILSVMLIFAFFQELVIAGIVENEWKRTCSRPKSNIVLLSAEEKKEQTIEIKEEVVGLTETSSQPKNEEDIEIIPIQEEEEEETETNFPEPPQDQESSPIENDSSP

SEQ ID NO: 52 - protein, 692 aa, Artificial sequence; identical to SEQ ID NO: 51
  Synthetic